European Patent Specification EP 3 678 682 B1, published April 1, 2026. Title: METHODS, COMPOSITIONS AND CELLS FOR PREPARING SURFACTANT PROTEIN D (SP-D). Applicant: Jan Susan Rosenbaum Frederick Gyapon Quast Matthias Kaup Lars Stockl. The sequence listing filed with the application follows.

SEQUENCE LISTING (10 sequences)

SEQ ID NO: 1 - DNA, 1150 bp, homo sapiens
aagcttgccaccatgctgctgtttctgctgagcgccctggtgctgctgacacagcctctgggctatctggaagccgagatgaagacctacagccaccggaccatgcccagcgcctgtaccctcgtgatgtgcagcagcgtggaaagcggcctgcctggcagagatggcagggatggaagagagggccccagaggcgagaagggcgatcctggactgcctggcgctgcagggcaggctggaatgcctggacaggctggacctgtgggccccaagggcgataatggctctgtgggagagcctggccctaagggggatacaggcccttctggacctcctggaccacctggcgtgccaggacctgctggaagagaaggacctctgggcaagcagggcaacatcggccctcagggaaagccaggaccaaagggcgaggccggacccaaaggcgaagtgggagcacctggcatgcagggaagtgccggcgctagaggactggctggcccaaaaggcgaaaggggagtgcctggcgaaagaggcgtgcccggaaatactggcgccgctggatctgctggcgccatgggacctcagggatctccaggcgcaagaggccctccaggcctgaaaggcgacaaaggcatccccggcgataagggcgctaagggcgaatccggcctgccagatgtggccagcctgagacagcaggtggaagctctccagggccaggtgcagcatctccaggctgccttcagccagtacaagaaggtggaactgttccccaacggccagagcgtgggcgagaagatctttaagaccgccggcttcgtgaagcccttcaccgaggctcagctgctgtgtacccaggctggcggacagctggcctctcctagatctgccgccgaaaatgccgctctccagcagctggtggtggccaagaatgaggccgccttcctgagcatgaccgacagcaagaccgagggcaagttcacctaccccaccggcgagtccctggtgtacagcaattgggcccctggcgagcccaacgatgatggcggctctgaggactgcgtggaaatcttcaccaacggcaagtggaacgaccgggcctgtggcgagaaaagactggtcgtgtgcgagttctgaagggtctaga

SEQ ID NO: 2 - DNA, 1138 bp, homo sapiens
gccaccatgctgctgtttctgctgagcgccctggtgctgctgacacagcctctgggctatctggaagccgagatgaagacctacagccaccggaccatgcccagcgcctgtaccctcgtgatgtgcagcagcgtggaaagcggcctgcctggcagagatggcagggatggaagagagggccccagaggcgagaagggcgatcctggactgcctggcgctgcagggcaggctggaatgcctggacaggctggacctgtgggccccaagggcgataatggctctgtgggagagcctggccctaagggggatacaggcccttctggacctcctggaccacctggcgtgccaggacctgctggaagagaaggacctctgggcaagcagggcaacatcggccctcagggaaagccaggaccaaagggcgaggccggacccaaaggcgaagtgggagcacctggcatgcagggaagtgccggcgctagaggactggctggcccaaaaggcgaaaggggagtgcctggcgaaagaggcgtgcccggaaatactggcgccgctggatctgctggcgccatgggacctcagggatctccaggcgcaagaggccctccaggcctgaaaggcgacaaaggcatccccggcgataagggcgctaagggcgaatccggcctgccagatgtggccagcctgagacagcaggtggaagctctccagggccaggtgcagcatctccaggctgccttcagccagtacaagaaggtggaactgttccccaacggccagagcgtgggcgagaagatctttaagaccgccggcttcgtgaagcccttcaccgaggctcagctgctgtgtacccaggctggcggacagctggcctctcctagatctgccgccgaaaatgccgctctccagcagctggtggtggccaagaatgaggccgccttcctgagcatgaccgacagcaagaccgagggcaagttcacctaccccaccggcgagtccctggtgtacagcaattgggcccctggcgagcccaacgatgatggcggctctgaggactgcgtggaaatcttcaccaacggcaagtggaacgaccgggcctgtggcgagaaaagactggtcgtgtgcgagttctgaaggg

SEQ ID NO: 3 - DNA, 60 bp, homo sapiens
atgctgctgtttctgctgagcgccctggtgctgctgacacagcctctgggctatctggaa

SEQ ID NO: 4 - protein, 375 aa, homo sapiens
MLLFLLSALVLLTQPLGYLEAEMKTYSHRTMPSACTLVMCSSVESGLPGRDGRDGREGPRGEKGDPGLPGAAGQAGMPGQAGPVGPKGDNGSVGEPGPKGDTGPSGPPGPPGVPGPAGREGPLGKQGNIGPQGKPGPKGEAGPKGEVGAPGMQGSAGARGLAGPKGERGVPGERGVPGNTGAAGSAGAMGPQGSPGARGPPGLKGDKGIPGDKGAKGESGLPDVASLRQQVEALQGQVQHLQAAFSQYKKVELFPNGQSVGEKIFKTAGFVKPFTEAQLLCTQAGGQLASPRSAAENAALQQLVVAKNEAAFLSMTDSKTEGKFTYPTGESLVYSNWAPGEPNDDGGSEDCVEIFTNGKWNDRACGEKRLVVCEF

SEQ ID NO: 5 - protein, 20 aa, homo sapiens
MLLFLLSALVLLTQPLGYLE

SEQ ID NO: 6 - DNA, 1153 bp, homo sapiens
aagcttgccaccatggcctgccccggatttctgtgggccctcgtgatcagcacctgtctggaattcagcatggccgccgagatgaagacctacagccaccggacaatgcccagcgcctgcaccctcgtgatgtgcagctctgtggaaagcggcctgcccggcagagatggcagggatggaagagagggacccagaggcgagaagggcgatcctggactgcctggcgctgcagggcaggctggaatgcctggacaggctggacctgtgggccccaagggcgataatggctctgtgggagagcctggccctaagggggatacaggcccttctggacctcctggaccacctggcgtgccaggacctgctggaagagaaggacctctgggcaagcagggcaacatcggccctcagggaaagccaggaccaaagggcgaggccggacccaaaggcgaagtgggagcacctggcatgcagggaagtgccggcgctagaggactggctggcccaaaaggcgaaaggggagtgcctggcgaaagaggcgtgcccggaaatactggcgccgctggatctgctggcgccatgggacctcagggatctccaggcgcaagaggccctccaggcctgaaaggcgacaaaggcatccccggcgataagggcgctaagggcgaatccggcctgccagatgtggccagcctgagacagcaggtggaagctctccagggccaggtgcagcatctccaggctgccttcagccagtacaagaaggtggaactgttccccaacggccagagcgtgggcgagaagatctttaagaccgccggcttcgtgaagcccttcaccgaggctcagctgctgtgtacccaggctggcggacagctggcctctcctagatctgccgccgaaaatgccgctctccagcagctggtggtggccaagaatgaggccgccttcctgagcatgaccgacagcaagaccgagggcaagttcacctaccccaccggcgagtccctggtgtacagcaattgggcccctggcgagcccaacgatgatggcggctctgaggactgcgtggaaatcttcaccaacggcaagtggaacgaccgggcctgtggcgagaaaagactggtcgtgtgcgagttctgaagggtctaga

SEQ ID NO: 7 - DNA, 1141 bp, homo sapiens
gccaccatggcctgccccggatttctgtgggccctcgtgatcagcacctgtctggaattcagcatggccgccgagatgaagacctacagccaccggacaatgcccagcgcctgcaccctcgtgatgtgcagctctgtggaaagcggcctgcccggcagagatggcagggatggaagagagggacccagaggcgagaagggcgatcctggactgcctggcgctgcagggcaggctggaatgcctggacaggctggacctgtgggccccaagggcgataatggctctgtgggagagcctggccctaagggggatacaggcccttctggacctcctggaccacctggcgtgccaggacctgctggaagagaaggacctctgggcaagcagggcaacatcggccctcagggaaagccaggaccaaagggcgaggccggacccaaaggcgaagtgggagcacctggcatgcagggaagtgccggcgctagaggactggctggcccaaaaggcgaaaggggagtgcctggcgaaagaggcgtgcccggaaatactggcgccgctggatctgctggcgccatgggacctcagggatctccaggcgcaagaggccctccaggcctgaaaggcgacaaaggcatccccggcgataagggcgctaagggcgaatccggcctgccagatgtggccagcctgagacagcaggtggaagctctccagggccaggtgcagcatctccaggctgccttcagccagtacaagaaggtggaactgttccccaacggccagagcgtgggcgagaagatctttaagaccgccggcttcgtgaagcccttcaccgaggctcagctgctgtgtacccaggctggcggacagctggcctctcctagatctgccgccgaaaatgccgctctccagcagctggtggtggccaagaatgaggccgccttcctgagcatgaccgacagcaagaccgagggcaagttcacctaccccaccggcgagtccctggtgtacagcaattgggcccctggcgagcccaacgatgatggcggctctgaggactgcgtggaaatcttcaccaacggcaagtggaacgaccgggcctgtggcgagaaaagactggtcgtgtgcgagttctgaaggg

SEQ ID NO: 8 - DNA, 63 bp, homo sapiens
atggcctgccccggatttctgtgggccctcgtgatcagcacctgtctggaattcagcatggcc

SEQ ID NO: 9 - protein, 376 aa, homo sapiens
MACPGFLWALVISTCLEFSMAAEMKTYSHRTMPSACTLVMCSSVESGLPGRDGRDGREGPRGEKGDPGLPGAAGQAGMPGQAGPVGPKGDNGSVGEPGPKGDTGPSGPPGPPGVPGPAGREGPLGKQGNIGPQGKPGPKGEAGPKGEVGAPGMQGSAGARGLAGPKGERGVPGERGVPGNTGAAGSAGAMGPQGSPGARGPPGLKGDKGIPGDKGAKGESGLPDVASLRQQVEALQGQVQHLQAAFSQYKKVELFPNGQSVGEKIFKTAGFVKPFTEAQLLCTQAGGQLASPRSAAENAALQQLVVAKNEAAFLSMTDSKTEGKFTYPTGESLVYSNWAPGEPNDDGGSEDCVEIFTNGKWNDRACGEKRLVVCEF

SEQ ID NO: 10 - protein, 21 aa, homo sapiens
MACPGFLWALVISTCLEFSMA